European Patent Specification EP 3 908 304 B1, published April 10, 2024. Title: COMPOSIZIONI COMPRENDENTI UN PEPTIDE IN GRADO DI STIMOLARE LA VIA DEL SEGNALE GPRC6A-DIPENDENTE. Applicant: IBSA IBSA    Fondazione Foresta. The sequence listing filed with the application follows.

SEQUENCE LISTING (1 sequence)

SEQ ID NO: 1 - protein, 16 aa, Artificial Sequence
  Synthetic peptide
NMYLPPVPPPPVVPTF